European Patent Specification EP 3 638 204 B1, published June 5, 2024. Title: Method of Alleviating Knee Pain. Applicant: Kumagai, Yoshinari. The sequence listing filed with the application follows.

SEQUENCE LISTING (1 sequence)

SEQ ID NO: 1 - protein, 23 aa, Artificial sequence
  Synthetic peptide sequence
TDLQERGDNDISPFSGDGQPFKD